European Patent Application EP 4 620 974 A1, published September 24, 2025. Title: ANTI-AFP/HLA02 TCR-LIKE ANTIBODY AND USE THEREOF. Applicant: Oricell Therapeutics Co.,Ltd. The sequence listing filed with the application follows.

SEQUENCE LISTING (150 sequences)

SEQ ID NO: 1 - DNA, 363 bp, synthetic construct
  misc_feature 1..363: note = 1B3 antibody nucleotide sequence
  source 1..363: mol_type = other DNA
gaggtgcagctggtggagagcggtggtggtctcgtgcagcccggcggtagtctgcgcctcagctgtgccgccagcggttttacctttagcaactatgtgatgggctggtttcgccaagcccccggcaaaggtcgcgaactggtggccaccattagcccaagcggtggcagcaccttttacccagatagcgtggaaggccgcttcaccatcagccgcgataacgccaagcgcatggtgtatctgcagatgaacagtctgcgcgccgaggacaccgccgtgtattattgtgccgccaaagatatctatcgcccagccctggattacgattactggggccaaggcacccaagtgaccgtgagcagc

SEQ ID NO: 2 - DNA, 372 bp, synthetic construct
  misc_feature 1..372: note = 1C4 antibody nucleotide sequence
  source 1..372: mol_type = other DNA
gaggtgcagctggtggagagcggtggtggtctcgtgcagcccggcggtagtctgcgcctcagctgtgccgccagcggtcgcacctttagccgctatgccatgggctggtttcgccaagcccccggcaaaggtcgcgaactggtggccgccatttcccgcacgggcggtagcacctactacccagatagcgtggaaggccgcttcaccatcagccgcgataacgccaagcgcatggtgtatctgcagatgaacagtctgcgcgccgaggacaccgccgtgtattattgtgccgccgatctgtattatggcccaatcatcaccgaaggcaactacgattactggggccaaggcacccaagtgaccgtgagcagc

SEQ ID NO: 3 - DNA, 372 bp, synthetic construct
  misc_feature 1..372: note = 1C11 antibody nucleotide sequence
  source 1..372: mol_type = other DNA
gaggtgcagctggtggagagcggtggtggtctcgtgcagcccggcggtagtctgcgcctcagctgtgccgccagcggtcgcacccttagccgctatgccatgggctggtttcgccaagcccccggcaaaggtcgcgaactggtggccgccatttcccgcacgggcggtagcacctactacccagatagcgtggaaggccgcttcaccatcagccgcgataacgccaagcgcatggtgtatctgcagatgaacagtctgcgcgccgaggacaccgccgtgtattattgtgccgccgatctgtattatggcccaatcatcaccgaaggcaactacgattactggggccaaggcacccaagtgaccgtgagcagc

SEQ ID NO: 4 - DNA, 372 bp, synthetic construct
  misc_feature 1..372: note = 1D12 antibody nucleotide sequence
  source 1..372: mol_type = other DNA
gaggtgcagctggtggagagcggtggtggtctcgtgcagcccggcggtagtctgcgcctcagctgtgccgccagcggtcgcacccttagcccatatgccatgggctggtttcgccaagcccccggcaaaggtcgcgaactggtggccgccatttcccgcacgggcggtagcacctactacccagatagcgtggaaggccgcttcaccatcagccgcgataacgccaagcgcatggtgtatctgcagatgaacagtctgcgcgccgaggacaccgccgtgtattattgtgccgccgatctgtattatggcccaatcatcaccgaaggcaactacaattactggggccaaggcacccaagtgaccgtgagcagc

SEQ ID NO: 5 - DNA, 363 bp, synthetic construct
  misc_feature 1..363: note = 2F9 antibody nucleotide sequence
  source 1..363: mol_type = other DNA
gaggtgcagctggtggagagcggtggtggtctcgtgcagcccggcggtagtctgcgcctcagctgtgccgccagcggtcgcatccttagccgctatgccatgggctggtttcgccaagcccccggcaaaggtcgcgaactggtggccaccattagcgcccgcggtagcagcacctattacccagatagcgtggaaggccgcttcaccatcagccgcgataacgccaagcgcatggtgtatctgcagatgaacagtctgcgcgccgaggacaccgccgtgtattattgtgccgccaacgatatcacctatacccaggccacctacgattactggggccaaggcacccaagtgaccgtgagcagc

SEQ ID NO: 6 - DNA, 372 bp, synthetic construct
  misc_feature 1..372: note = No.3 antibody nucleotide sequence
  source 1..372: mol_type = other DNA
gaggtgcagctggtggagagcggtggtggtctcgtgcagcccggcggtagtctgcgcctcagctgtgccgccagcggtcgcacctttagcagctatgccatgggctggtttcgccaagcccccggcaaaggtcgcgaactggtggccgccatttcccgcacgggcggtagcacctactacccagatagcgtggaaggccgcttcaccatcagccgcgataacgccaagcgcatggtgtatctgcagatgaacagtctgcgcgccgaggacaccgccgtgtattattgtgccgccgatctgtattatggcccaatcatcaccgaaggcaactacgattactggggccaaggcacccaagtgaccgtgagcagc

SEQ ID NO: 7 - DNA, 372 bp, synthetic construct
  misc_feature 1..372: note = No.4 antibody nucleotide sequence
  source 1..372: mol_type = other DNA
gaggtgcagctggtggagagcggtggtggtctcgtgcagcccggcggtagtctgcgcctcagctgtgccgccagcggtagcatctttagcacctatgccatgggctggtttcgccaagcccccggcaaaggtcgcgaactggtggccgccatttcccgcacgggcggtagcacctactacccagatagcgtggaaggccgcttcaccatcagccgcgataacgccaagcgcatggtgtatctgcagatgaacagtctgcgcgccgaggacaccgccgtgtattattgtgccgccgatctgtattatggcccaatcatcaccgaaggcaactacgattactggggccaaggcacccaagtgaccgtgagcagc

SEQ ID NO: 8 - DNA, 372 bp, synthetic construct
  misc_feature 1..372: note = No.7 antibody nucleotide sequence
  source 1..372: mol_type = other DNA
gaggtgcagctggtggagagcggtggtggtctcgtgcagcccggcggtagtctgcgcctcagctgtgccgccagcggtcgcacccttagccgctatgccatgggctggtttcgccaagcccccggcaaaggtcgcgaactggtggccgccatttcccgcacgggcggtagcacctactacccagatagcgtggaaggccgcttcaccatcagccgcgataacgccaagcgcatggtgtatctgcagatgaacagtctgcgcgccgaggacaccgccgtgtattattgtgccgccgatctgtattatggcccaatcatcaccgaaggcaactacaattactggggccaaggcacccaagtgaccgtgagcagc

SEQ ID NO: 9 - DNA, 372 bp, synthetic construct
  misc_feature 1..372: note = No.8 antibody nucleotide sequence
  source 1..372: mol_type = other DNA
gaggtgcagctggtggagagcggtggtggtctcgtgcagcccggcggtagtctgcgcctcagctgtgccgccagcggtgatacccttagccgctatgccatgggctggtttcgccaagcccccggcaaaggtcgcgaactggtggccgccatttcccgcacgggcggtagcacctactacccagatagcgtggaaggccgcttcaccatcagccgcgataacgccaagcgcatggtgtatctgcagatgaacagtctgcgcgccgaggacaccgccgtgtattattgtgccgccgatctgtattatggcccaatcatcaccgaaggcaactacaattactggggccaaggcacccaagtgaccgtgagcagc

SEQ ID NO: 10 - DNA, 363 bp, synthetic construct
  misc_feature 1..363: note = No.15 antibody nucleotide sequence
  source 1..363: mol_type = other DNA
gaggtgcagctggtggagagcggtggtggtctcgtgcagcccggcggtagtctgcgcctcagctgtgccgccagcggtctgatctttagccgctattatatgggctggtttcgccaagcccccggcaaaggtcgcgaactggtggccggcattacccgcagcggtggcggcacctattacccagatagcgtggaaggccgcttcaccatcagccgcgataacgccaagcgcatggtgtatctgcagatgaacagtctgcgcgccgaggacaccgccgtgtattattgtgccgccgaaccagccggctattatcaggaaaactacgattactggggccaaggcacccaagtgaccgtgagcagc

SEQ ID NO: 11 - DNA, 360 bp, synthetic construct
  misc_feature 1..360: note = No.17 antibody nucleotide sequence
  source 1..360: mol_type = other DNA
gaggtgcagctggtggagagcggtggtggtctcgtgcagcccggcggtagtctgcgcctcagctgtgccgccagcggtttgatctttagcaacgattatatgggctggtttcgccaagcccccggcaaaggtcgcgaactggtggccaccattagcacccgcggtggcacctactacccacataacgtggaaggacgcttcatcatcatccgcgataacgacaagcgcatggtgtatctgctgatgaacagtctgcgcgccgaggacaccgccgtgtattattgtgccgccgatagcatcatcggctatgccacagaatactattactgctgccaaggcagcaaagtgaccgtgagcagc

SEQ ID NO: 12 - DNA, 363 bp, synthetic construct
  misc_feature 1..363: note = No.24 antibody nucleotide sequence
  source 1..363: mol_type = other DNA
gaggtgcagctggtggagagcggtggtggtctcgtgcagcccggcggtagtctgcgcctcagctgtgccgccagcggtcgcatccttagccgctatgccatgggctggtttcgccaagcccccggcaaaggtcgcgaactggtggccaccattagcgccagcggtggcaccacctattacccagatagcgtggaaggccgcttcaccatcagccgcgataacgccaagcgcatggtgtatctgcagatgaacagtctgcgcgccgaggacaccgccgtgtattattgtgccgccgccgatatctatagcagcgatgccgattacaattactggggccaaggcacccaagtgaccgtgagcagc

SEQ ID NO: 13 - DNA, 372 bp, synthetic construct
  misc_feature 1..372: note = No.29 antibody nucleotide sequence
  source 1..372: mol_type = other DNA
gaggtgcagctggtggagagcggtggtggtctcgtgcagcccggcggtagtctgcgcctcagctgtgccgccagcggtaacacctttagcagctatgccatgggctggtttcgccaagcccccggcaaaggtcgcgaactggtggccgccatttcccgcacgggcggtagcacctactacccagatagcgtggaaggccgcttcaccatcagccgcgataacgccaagcgcatggtgtatctgcatatgaacagtctgcgcgccgaggacaccgccgtgtattattgtgccgccgatctgtattatggcccaatcatcaccgaaggcaactacaattactggggccaaggcacccaagtgaccgtgagcagc

SEQ ID NO: 14 - protein, 7 aa, synthetic construct
  REGION 1..7: note = 1B3 HCDR1 (IMGT)
GFTFSNY

SEQ ID NO: 15 - protein, 8 aa, synthetic construct
  REGION 1..8: note = 1B3 HCDR2 (IMGT)
ISPSGGST

SEQ ID NO: 16 - protein, 14 aa, synthetic construct
  REGION 1..14: note = 1B3 HCDR3 (IMGT)
AAKDIYRPALDYDY

SEQ ID NO: 17 - protein, 5 aa, synthetic construct
  REGION 1..5: note = 1B3 HCDR1 (Kabat)
NYVMG

SEQ ID NO: 18 - protein, 17 aa, synthetic construct
  REGION 1..17: note = 1B3 HCDR2 (Kabat)
TISPSGGSTFYPDSVEG

SEQ ID NO: 19 - protein, 12 aa, synthetic construct
  REGION 1..12: note = 1B3 HCDR3 (Kabat)
KDIYRPALDYDY

SEQ ID NO: 20 - protein, 7 aa, synthetic construct
  REGION 1..7: note = 1C4 HCDR1 (IMGT)
GRTFSRY

SEQ ID NO: 21 - protein, 8 aa, synthetic construct
  REGION 1..8: note = 1C4 HCDR2 (IMGT); 1C11 HCDR2 (IMGT); 1D12 HCDR2 (IMGT); No.3HCDR2 (IMGT); No.4 HCDR2 (IMGT); No.7 HCDR2 (IMGT); No.8 HCDR2 (IMGT); No.29 HCDR2 (IMGT)
ISRTGGST

SEQ ID NO: 22 - protein, 17 aa, synthetic construct
  REGION 1..17: note = 1C4 HCDR3 (IMGT); 1C11 HCDR3 (IMGT); No.3 HCDR3 (IMGT);No.4 HCDR3 (IMGT)
AADLYYGPIITEGNYDY

SEQ ID NO: 23 - protein, 5 aa, synthetic construct
  REGION 1..5: note = 1C4 HCDR1 (Kabat); 1C11 HCDR1 (Kabat); 2F9 HCDR1 (Kabat); No.7 HCDR1 (Kabat); No.8 HCDR1 (Kabat); No.24 HCDR1 (Kabat)
RYAMG

SEQ ID NO: 24 - protein, 17 aa, synthetic construct
  REGION 1..17: note = 1C4 HCDR2 (Kabat); 1C11 HCDR2 (Kabat); 1D12 HCDR2 (Kabat); No.3 HCDR2 (Kabat); No.4 HCDR2 (Kabat); No.7 HCDR2 (Kabat); No.8 HCDR2 (Kabat); No.29 HCDR2 (Kabat)
AISRTGGSTYYPDSVEG

SEQ ID NO: 25 - protein, 15 aa, synthetic construct
  REGION 1..15: note = 1C4 HCDR3 (Kabat); 1C11 HCDR3 (Kabat); No.3 HCDR3 (Kabat); No.4 HCDR3 (Kabat)
DLYYGPIITEGNYDY

SEQ ID NO: 26 - protein, 7 aa, synthetic construct
  REGION 1..7: note = 1C11 HCDR1 (IMGT); No.7 HCDR1 (IMGT)
GRTLSRY

SEQ ID NO: 27 - protein, 7 aa, synthetic construct
  REGION 1..7: note = 1D12 HCDR1 (IMGT)
GRTLSPY

SEQ ID NO: 28 - protein, 17 aa, synthetic construct
  REGION 1..17: note = 1D12 HCDR3 (IMGT); No.7 HCDR3 (IMGT); No.8 HCDR3 (IMGT); No.29 HCDR3 (IMGT)
AADLYYGPIITEGNYNY

SEQ ID NO: 29 - protein, 5 aa, synthetic construct
  REGION 1..5: note = 1D12 HCDR1 (Kabat)
PYAMG

SEQ ID NO: 30 - protein, 15 aa, synthetic construct
  REGION 1..15: note = 1D12 HCDR3 (Kabat); No.7 HCDR3 (Kabat); No.8 HCDR3 (Kabat); No.29 HCDR3 (Kabat)
DLYYGPIITEGNYNY

SEQ ID NO: 31 - protein, 7 aa, synthetic construct
  REGION 1..7: note = 2F9 HCDR1 (IMGT); No.24 HCDR1 (IMGT)
GRILSRY

SEQ ID NO: 32 - protein, 8 aa, synthetic construct
  REGION 1..8: note = 2F9 HCDR2 (IMGT)
ISARGSST

SEQ ID NO: 33 - protein, 14 aa, synthetic construct
  REGION 1..14: note = 2F9 HCDR3 (IMGT)
AANDITYTQATYDY

SEQ ID NO: 34 - protein, 17 aa, synthetic construct
  REGION 1..17: note = 2F9 HCDR2 (Kabat)
TISARGSSTYYPDSVEG

SEQ ID NO: 35 - protein, 12 aa, synthetic construct
  REGION 1..12: note = 2F9 HCDR3 (Kabat)
NDITYTQATYDY

SEQ ID NO: 36 - protein, 7 aa, synthetic construct
  REGION 1..7: note = No.3 HCDR1 (IMGT)
GRTFSSY

SEQ ID NO: 37 - protein, 5 aa, synthetic construct
  REGION 1..5: note = No.3 HCDR1 (Kabat); No.29HCDR1 (Kabat)
SYAMG

SEQ ID NO: 38 - protein, 7 aa, synthetic construct
  REGION 1..7: note = No.4 HCDR1 (IMGT)
GSIFSTY

SEQ ID NO: 39 - protein, 5 aa, synthetic construct
  REGION 1..5: note = No.4 HCDR1 (Kabat)
TYAMG

SEQ ID NO: 40 - protein, 7 aa, synthetic construct
  REGION 1..7: note = No.8 HCDR1 (IMGT)
GDTLSRY

SEQ ID NO: 41 - protein, 7 aa, synthetic construct
  REGION 1..7: note = No.15 HCDR1 (IMGT)
GLIFSRY

SEQ ID NO: 42 - protein, 8 aa, synthetic construct
  REGION 1..8: note = No.15 HCDR2 (IMGT)
ITRSGGGT

SEQ ID NO: 43 - protein, 14 aa, synthetic construct
  REGION 1..14: note = No.15 HCDR3 (IMGT)
AAEPAGYYQENYDY

SEQ ID NO: 44 - protein, 5 aa, synthetic construct
  REGION 1..5: note = No.15HCDR1 (Kabat)
RYYMG

SEQ ID NO: 45 - protein, 17 aa, synthetic construct
  REGION 1..17: note = No.15HCDR2 (Kabat)
GITRSGGGTYYPDSVEG

SEQ ID NO: 46 - protein, 12 aa, synthetic construct
  REGION 1..12: note = No.15HCDR3 (Kabat)
EPAGYYQENYDY

SEQ ID NO: 47 - protein, 7 aa, synthetic construct
  REGION 1..7: note = No.17 HCDR1 (IMGT)
GLIFSND

SEQ ID NO: 48 - protein, 8 aa, synthetic construct
  REGION 1..8: note = No.17 HCDR2 (IMGT)
ISTRGGTY

SEQ ID NO: 49 - protein, 14 aa, synthetic construct
  REGION 1..14: note = No.17 HCDR3 (IMGT)
AADSIIGYATEYYY

SEQ ID NO: 50 - protein, 5 aa, synthetic construct
  REGION 1..5: note = No.17 HCDR1 (Kabat)
NDYMG

SEQ ID NO: 51 - protein, 16 aa, synthetic construct
  REGION 1..16: note = No.17 HCDR2 (Kabat)
TISTRGGTYYPHNVEG

SEQ ID NO: 52 - protein, 12 aa, synthetic construct
  REGION 1..12: note = No.17 HCDR3 (Kabat)
DSIIGYATEYYY

SEQ ID NO: 53 - protein, 8 aa, synthetic construct
  REGION 1..8: note = No.24 HCDR2 (IMGT)
ISASGGTT

SEQ ID NO: 54 - protein, 14 aa, synthetic construct
  REGION 1..14: note = No.24 HCDR3 (IMGT)
AAADIYSSDADYNY

SEQ ID NO: 55 - protein, 17 aa, synthetic construct
  REGION 1..17: note = No.24 HCDR2 (Kabat)
TISASGGTTYYPDSVEG

SEQ ID NO: 56 - protein, 12 aa, synthetic construct
  REGION 1..12: note = No.24 HCDR3 (Kabat)
ADIYSSDADYNY

SEQ ID NO: 57 - protein, 7 aa, synthetic construct
  REGION 1..7: note = No.29 HCDR1 (IMGT)
GNTFSSY

SEQ ID NO: 58 - protein, 30 aa, synthetic construct
  REGION 1..30: note = 1B3 H-FR1 (Kabat)
EVQLVESGGGLVQPGGSLRLSCAASGFTFS

SEQ ID NO: 59 - protein, 30 aa, synthetic construct
  REGION 1..30: note = 1C4 H-FR1 (Kabat); No.3 H-FR1 (Kabat)
EVQLVESGGGLVQPGGSLRLSCAASGRTFS

SEQ ID NO: 60 - protein, 30 aa, synthetic construct
  REGION 1..30: note = 1C11 H-FR1 (Kabat); 1D12 H-FR1 (Kabat); No.7 H-FR1 (Kabat)
EVQLVESGGGLVQPGGSLRLSCAASGRTLS

SEQ ID NO: 61 - protein, 30 aa, synthetic construct
  REGION 1..30: note = 2F9 H-FR1 (Kabat); No.24 H-FR1 (Kabat)
EVQLVESGGGLVQPGGSLRLSCAASGRILS

SEQ ID NO: 62 - protein, 30 aa, synthetic construct
  REGION 1..30: note = No.4 H-FR1 (Kabat)
EVQLVESGGGLVQPGGSLRLSCAASGSIFS

SEQ ID NO: 63 - protein, 30 aa, synthetic construct
  REGION 1..30: note = No.8 H-FR1 (Kabat)
EVQLVESGGGLVQPGGSLRLSCAASGDTLS

SEQ ID NO: 64 - protein, 30 aa, synthetic construct
  REGION 1..30: note = No.15 H-FR1 (Kabat); No.17 H-FR1 (Kabat)
EVQLVESGGGLVQPGGSLRLSCAASGLIFS

SEQ ID NO: 65 - protein, 30 aa, synthetic construct
  REGION 1..30: note = No.29 H-FR1 (Kabat)
EVQLVESGGGLVQPGGSLRLSCAASGNTFS

SEQ ID NO: 66 - protein, 14 aa, synthetic construct
  REGION 1..14: note = 1B3 H-FR2 (Kabat); 1C4 H-FR2 (Kabat); 1C11 H-FR2 (Kabat); 1D12 H-FR2 (Kabat); 2F9 H-FR2 (Kabat); No.3 H-FR2 (Kabat); No.4 H-FR2 (Kabat); No.7 H-FR2 (Kabat); No.8 H-FR2 (Kabat); No.15 H-FR2 (Kabat); No.17 H-FR2 (Kabat); No.24 H-FR2 (Kabat); No.29 H-FR2 (Kabat)
WFRQAPGKGRELVA

SEQ ID NO: 67 - protein, 32 aa, synthetic construct
  REGION 1..32: note = 1B3 H-FR3 (Kabat); 1C4 H-FR3 (Kabat); 1C11 H-FR3 (Kabat); 1D12 H-FR3 (Kabat); 2F9 H-FR3 (Kabat); No.3 H-FR3 (Kabat); No.4 H-FR3 (Kabat); No.7 H-FR3 (Kabat); No.8 H-FR3 (Kabat); No.15 H-FR3 (Kabat); No.24 H-FR3 (Kabat)
RFTISRDNAKRMVYLQMNSLRAEDTAVYYCAA

SEQ ID NO: 68 - protein, 32 aa, synthetic construct
  REGION 1..32: note = No.17 H-FR3 (Kabat)
RFIIIRDNDKRMVYLLMNSLRAEDTAVYYCAA

SEQ ID NO: 69 - protein, 32 aa, synthetic construct
  REGION 1..32: note = No.29 H-FR3 (Kabat)
RFTISRDNAKRMVYLHMNSLRAEDTAVYYCAA

SEQ ID NO: 70 - protein, 11 aa, synthetic construct
  REGION 1..11: note = 1B3 H-FR4 (Kabat); 1C4 H-FR4 (Kabat); 1C11 H-FR4 (Kabat); 1D12 H-FR4 (Kabat); 2F9 H-FR4 (Kabat); No.3 H-FR4 (Kabat); No.4 H-FR4 (Kabat); No.7 H-FR4 (Kabat); No.8 H-FR4 (Kabat); No.15 H-FR4 (Kabat); No.24 H-FR4 (Kabat); No.29 H-FR4 (Kabat)
WGQGTQVTVSS

SEQ ID NO: 71 - protein, 11 aa, synthetic construct
  REGION 1..11: note = No.17 H-FR4 (Kabat)
CCQGSKVTVSS

SEQ ID NO: 72 - protein, 121 aa, synthetic construct
  REGION 1..121: note = 1B3 antibody amino acid sequence
EVQLVESGGGLVQPGGSLRLSCAASGFTFSNYVMGWFRQAPGKGRELVATISPSGGSTFYPDSVEGRFTISRDNAKRMVYLQMNSLRAEDTAVYYCAAKDIYRPALDYDYWGQGTQVTVSS

SEQ ID NO: 73 - protein, 124 aa, synthetic construct
  REGION 1..124: note = 1C4 antibody amino acid sequence
EVQLVESGGGLVQPGGSLRLSCAASGRTFSRYAMGWFRQAPGKGRELVAAISRTGGSTYYPDSVEGRFTISRDNAKRMVYLQMNSLRAEDTAVYYCAADLYYGPIITEGNYDYWGQGTQVTVSS

SEQ ID NO: 74 - protein, 124 aa, synthetic construct
  REGION 1..124: note = 1C11 antibody amino acid sequence
EVQLVESGGGLVQPGGSLRLSCAASGRTLSRYAMGWFRQAPGKGRELVAAISRTGGSTYYPDSVEGRFTISRDNAKRMVYLQMNSLRAEDTAVYYCAADLYYGPIITEGNYDYWGQGTQVTVSS

SEQ ID NO: 75 - protein, 124 aa, synthetic construct
  REGION 1..124: note = 1D12 antibody amino acid sequence
EVQLVESGGGLVQPGGSLRLSCAASGRTLSPYAMGWFRQAPGKGRELVAAISRTGGSTYYPDSVEGRFTISRDNAKRMVYLQMNSLRAEDTAVYYCAADLYYGPIITEGNYNYWGQGTQVTVSS

SEQ ID NO: 76 - protein, 121 aa, synthetic construct
  REGION 1..121: note = 2F9 antibody amino acid sequence
EVQLVESGGGLVQPGGSLRLSCAASGRILSRYAMGWFRQAPGKGRELVATISARGSSTYYPDSVEGRFTISRDNAKRMVYLQMNSLRAEDTAVYYCAANDITYTQATYDYWGQGTQVTVSS

SEQ ID NO: 77 - protein, 124 aa, synthetic construct
  REGION 1..124: note = No.3 antibody amino acid sequence
EVQLVESGGGLVQPGGSLRLSCAASGRTFSSYAMGWFRQAPGKGRELVAAISRTGGSTYYPDSVEGRFTISRDNAKRMVYLQMNSLRAEDTAVYYCAADLYYGPIITEGNYDYWGQGTQVTVSS

SEQ ID NO: 78 - protein, 124 aa, synthetic construct
  REGION 1..124: note = No.4 antibody amino acid sequence
EVQLVESGGGLVQPGGSLRLSCAASGSIFSTYAMGWFRQAPGKGRELVAAISRTGGSTYYPDSVEGRFTISRDNAKRMVYLQMNSLRAEDTAVYYCAADLYYGPIITEGNYDYWGQGTQVTVSS

SEQ ID NO: 79 - protein, 124 aa, synthetic construct
  REGION 1..124: note = No.7 antibody amino acid sequence
EVQLVESGGGLVQPGGSLRLSCAASGRTLSRYAMGWFRQAPGKGRELVAAISRTGGSTYYPDSVEGRFTISRDNAKRMVYLQMNSLRAEDTAVYYCAADLYYGPIITEGNYNYWGQGTQVTVSS

SEQ ID NO: 80 - protein, 124 aa, synthetic construct
  REGION 1..124: note = No.8 antibody amino acid sequence
EVQLVESGGGLVQPGGSLRLSCAASGDTLSRYAMGWFRQAPGKGRELVAAISRTGGSTYYPDSVEGRFTISRDNAKRMVYLQMNSLRAEDTAVYYCAADLYYGPIITEGNYNYWGQGTQVTVSS

SEQ ID NO: 81 - protein, 121 aa, synthetic construct
  REGION 1..121: note = No.15 antibody amino acid sequence
EVQLVESGGGLVQPGGSLRLSCAASGLIFSRYYMGWFRQAPGKGRELVAGITRSGGGTYYPDSVEGRFTISRDNAKRMVYLQMNSLRAEDTAVYYCAAEPAGYYQENYDYWGQGTQVTVSS

SEQ ID NO: 82 - protein, 120 aa, synthetic construct
  REGION 1..120: note = No.17 antibody amino acid sequence
EVQLVESGGGLVQPGGSLRLSCAASGLIFSNDYMGWFRQAPGKGRELVATISTRGGTYYPHNVEGRFIIIRDNDKRMVYLLMNSLRAEDTAVYYCAADSIIGYATEYYYCCQGSKVTVSS

SEQ ID NO: 83 - protein, 121 aa, synthetic construct
  REGION 1..121: note = No.24 antibody amino acid sequence
EVQLVESGGGLVQPGGSLRLSCAASGRILSRYAMGWFRQAPGKGRELVATISASGGTTYYPDSVEGRFTISRDNAKRMVYLQMNSLRAEDTAVYYCAAADIYSSDADYNYWGQGTQVTVSS

SEQ ID NO: 84 - protein, 124 aa, synthetic construct
  REGION 1..124: note = No.29 antibody amino acid sequence
EVQLVESGGGLVQPGGSLRLSCAASGNTFSSYAMGWFRQAPGKGRELVAAISRTGGSTYYPDSVEGRFTISRDNAKRMVYLHMNSLRAEDTAVYYCAADLYYGPIITEGNYNYWGQGTQVTVSS

SEQ ID NO: 85 - DNA, 729 bp, synthetic construct
  misc_feature 1..729: note = AB61 nucleotide sequence
  source 1..729: mol_type = other DNA
cagagcgtgctgacacagcctgcctccgtgtctggctctcctggccagtccatcaccatcagctgtaccggcaccagctccgacgtgggcggctacaattacgtgtcctggtatcagcagcatcccggcaaggcccccaagctgatgatctacgacgtgaacaaccggcccagcgaggtgtccaacagattcagcggcagcaagagcggcaacaccgccagcctgacaatcagcggactgcaggccgaggacgaggccgactactactgcagcagctacaccaccggcagcagagccgtgtttggcggaggcaccaagctgacagtgctgggcggtggcggtggctcgggcggtggtgggtcgggtggcggcggatctgaggtgcagctggtgcagtctggcgccgaagtgaagaagcctggcgagagcctgaccatctcctgcaaggccagcggctacagcttccccaactactggatcacctgggtgcgccagatgtccggcggaggcctggaatggatgggcagaatcgaccccggcgacagctacacaacctacaaccccagcttccagggccacgtgaccatcagcatcgacaagagcaccaataccgcctacctgcactggaacagcctgaaggcctccgacaccgccatgtactactgcgcccggtactatgtgtccctggtggatatctggggccagggcacactcgtgaccgtgtctagc

SEQ ID NO: 86 - protein, 243 aa, synthetic construct
  REGION 1..243: note = AB61 amino acid sequence
QSVLTQPASVSGSPGQSITISCTGTSSDVGGYNYVSWYQQHPGKAPKLMIYDVNNRPSEVSNRFSGSKSGNTASLTISGLQAEDEADYYCSSYTTGSRAVFGGGTKLTVLGGGGGSGGGGSGGGGSEVQLVQSGAEVKKPGESLTISCKASGYSFPNYWITWVRQMSGGGLEWMGRIDPGDSYTTYNPSFQGHVTISIDKSTNTAYLHWNSLKASDTAMYYCARYYVSLVDIWGQGTLVTVSS

SEQ ID NO: 87 - DNA, 708 bp, synthetic construct
  misc_feature 1..708: note = Fc nucleotide sequence
  source 1..708: mol_type = other DNA
gcggccgcagagcccaaatcttgtgacaaaactcacacatgcccaccgtgcccagcacctgaactcctggggggaccgtcagtcttcctcttccccccaaaacccaaggacaccctcatgatctcccggacccctgaggtcacatgcgtggtggtggacgtgagccacgaagaccctgaggtcaagttcaactggtacgtggacggcgtggaggtgcataatgccaagacaaagccgcgggaggagcagtacaacagcacgtaccgtgtggtcagcgtcctcaccgtcctgcaccaggactggctgaatggcaaggagtacaagtgcaaggtctccaacaaagccctcccagcccccatcgagaaaaccatctccaaagccaaagggcagccccgagaaccacaggtgtacaccctgcccccatcccgggatgagctgaccaagaaccaggtcagcctgacctgcctggtcaaaggcttctatcccagcgacatcgccgtggagtgggagagcaatgggcagccggagaacaactacaagaccacgcctcccgtgctggactccgacggctccttcttcctctacagcaagctcaccgtggacaagagcaggtggcagcaggggaacgtcttctcatgctccgtgatgcatgaggctctgcacaaccactacacgcagaagagcctctccctgtctcccggtaaatga

SEQ ID NO: 88 - protein, 236 aa, synthetic construct
  REGION 1..236: note = Fc amino acid sequence
  VARIANT 236: note = misc_feature - Xaa = any one kind of amino acid
AAAEPKSCDKTHTCPPCPAPELLGGPSVFLFPPKPKDTLMISRTPEVTCVVVDVSHEDPEVKFNWYVDGVEVHNAKTKPREEQYNSTYRVVSVLTVLHQDWLNGKEYKCKVSNKALPAPIEKTISKAKGQPREPQVYTLPPSRDELTKNQVSLTCLVKGFYPSDIAVEWESNGQPENNYKTTPPVLDSDGSFFLYSKLTVDKSRWQQGNVFSCSVMHEALHNHYTQKSLSLSPGKX

SEQ ID NO: 89 - DNA, 27 bp, synthetic construct
  misc_feature 1..27: note = human AFP158-166 gene
  source 1..27: mol_type = other DNA
ttcatgaacaaattcatttatgagata

SEQ ID NO: 90 - protein, 9 aa, synthetic construct
  REGION 1..9: note = human AFP158 polypeptide amino aicd sequence
FMNKFIYEI

SEQ ID NO: 91 - protein, 9 aa, synthetic construct
  REGION 1..9: note = human NY-Eso-1 157 polypeptide amino acid sequence
SLLMWITQC

SEQ ID NO: 92 - protein, 9 aa, synthetic construct
  REGION 1..9: note = IFI30 amino acid sequence
LLDVPTAAV

SEQ ID NO: 93 - protein, 10 aa, synthetic construct
  REGION 1..10: note = IFI30 amino acid sequence 2
LLLDVPTAAV

SEQ ID NO: 94 - protein, 11 aa, synthetic construct
  REGION 1..11: note = IFI30 amino acid sequence 3
LLLDVPTAAVQ

SEQ ID NO: 95 - protein, 12 aa, synthetic construct
  REGION 1..12: note = IFI30 amino acid sequence 4
LLLDVPTAAVQA

SEQ ID NO: 96 - protein, 9 aa, synthetic construct
  REGION 1..9: note = BTG2 amino acid sequence
TLWVDPYEV

SEQ ID NO: 97 - protein, 9 aa, synthetic construct
  REGION 1..9: note = BCR amino acid sequence
FLLDHLKRV

SEQ ID NO: 98 - protein, 13 aa, synthetic construct
  REGION 1..13: note = SSR1 amino acid sequence 1
VLFRGGPRGLLAV

SEQ ID NO: 99 - protein, 14 aa, synthetic construct
  REGION 1..14: note = SSR1 amino acid sequence 2
VLFRGGPRGLLAVA

SEQ ID NO: 100 - protein, 9 aa, synthetic construct
  REGION 1..9: note = PPP2R1B amino acid sequence
SLLPAIVEL

SEQ ID NO: 101 - protein, 9 aa, synthetic construct
  REGION 1..9: note = DDX5 amino acid sequence
YLLPAIVHI

SEQ ID NO: 102 - protein, 9 aa, synthetic construct
  REGION 1..9: note = CTSG amino acid sequence
FLLPTGAEA

SEQ ID NO: 103 - protein, 10 aa, synthetic construct
  REGION 1..10: note = CD247 amino acid sequence
LLDPKLCYLL

SEQ ID NO: 104 - protein, 10 aa, synthetic construct
  REGION 1..10: note = DMTN amino acid sequence
SLPHFHHPET

SEQ ID NO: 105 - protein, 10 aa, synthetic construct
  REGION 1..10: note = CALR amino acid sequence
MLLSVPLLLG

SEQ ID NO: 106 - protein, 11 aa, synthetic construct
  REGION 1..11: note = PIM1 amino acid sequence
LLYDMVCGDIP

SEQ ID NO: 107 - protein, 9 aa, synthetic construct
  REGION 1..9: note = HLA-E amino acid sequence
MVDGTLLLL

SEQ ID NO: 108 - protein, 10 aa, synthetic construct
  REGION 1..10: note = RPS6KB1 amino acid sequence
YMAPEILMRS

SEQ ID NO: 109 - protein, 10 aa, synthetic construct
  REGION 1..10: note = CSF2RA amino acid sequence
FIYNADLMNC

SEQ ID NO: 110 - protein, 11 aa, synthetic construct
  REGION 1..11: note = IL7 amino acid sequence
KQYESVLMVSI

SEQ ID NO: 111 - protein, 9 aa, synthetic construct
  REGION 1..9: note = human TERT540 polypeptide amino acid sequence
ILAKFLHWL

SEQ ID NO: 112 - protein, 781 aa, synthetic construct
  REGION 1..781: note = 1B3-CAR amino acid sequence
MALPVTALLLPLALLLHAARPEVQLVESGGGLVQPGGSLRLSCAASGFTFSNYVMGWFRQAPGKGRELVATISPSGGSTFYPDSVEGRFTISRDNAKRMVYLQMNSLRAEDTAVYYCAAKDIYRPALDYDYWGQGTQVTVSSTTTPAPRPPTPAPTIASQPLSLRPEACRPAAGGAVHTRGLDFACDIYIWAPLAGTCGVLLLSLVITLYCKRGRKKLLYIFKQPFMRPVQTTQEEDGCSCRFPEEEEGGCELRVKFSRSADAPAYQQGQNQLYNELNLGRREEYDVLDKRRGRDPEMGGKPRRKNPQEGLYNELQKDKMAEAYSEIGMKGERRRGKGHDGLYQGLSTATKDTYDALHMQALPPREGRGSLLTCGDVEENPGPMGAVLRSLLACSFCVLLRAEQKLISEEDLEPPTCSPQQFTCFTGEIDCIPVAWRCDGFTECEDHSDELNCPVCSESQFQCASGQCIDGALRCNGDANCQDKSDEKNCEVLCLIDQFRCANGQCIGKHKKCDHNVDCSDKSDELDCYPTEEPAPQATNTVGSVIGVIVTIFVSGTVYFICQRMLCPRMKGDGETMTNDYVVHGPASVPLGYVPHPSSLSGSLPGMSRGKSMISSLSIMGGSSGPPYDRAHVTGASSSSSSSTKGTYFPAILNPPPSPATERSHYTMEFGYSSNSPSTHRSYSYRPYSYRHFAPPTTPCSTDVCDSDYAPSRRMTSVATAKGYTSDLNYDSEPVPPPPTPRSQYLSAEENYESCPPSPYTERSYSHHLYPPPPSPCTDSS

SEQ ID NO: 113 - protein, 784 aa, synthetic construct
  REGION 1..784: note = 1C4-CAR amino acid sequence
MALPVTALLLPLALLLHAARPEVQLVESGGGLVQPGGSLRLSCAASGRTFSRYAMGWFRQAPGKGRELVAAISRTGGSTYYPDSVEGRFTISRDNAKRMVYLQMNSLRAEDTAVYYCAADLYYGPIITEGNYDYWGQGTQVTVSSTTTPAPRPPTPAPTIASQPLSLRPEACRPAAGGAVHTRGLDFACDIYIWAPLAGTCGVLLLSLVITLYCKRGRKKLLYIFKQPFMRPVQTTQEEDGCSCRFPEEEEGGCELRVKFSRSADAPAYQQGQNQLYNELNLGRREEYDVLDKRRGRDPEMGGKPRRKNPQEGLYNELQKDKMAEAYSEIGMKGERRRGKGHDGLYQGLSTATKDTYDALHMQALPPREGRGSLLTCGDVEENPGPMGAVLRSLLACSFCVLLRAEQKLISEEDLEPPTCSPQQFTCFTGEIDCIPVAWRCDGFTECEDHSDELNCPVCSESQFQCASGQCIDGALRCNGDANCQDKSDEKNCEVLCLIDQFRCANGQCIGKHKKCDHNVDCSDKSDELDCYPTEEPAPQATNTVGSVIGVIVTIFVSGTVYFICQRMLCPRMKGDGETMTNDYVVHGPASVPLGYVPHPSSLSGSLPGMSRGKSMISSLSIMGGSSGPPYDRAHVTGASSSSSSSTKGTYFPAILNPPPSPATERSHYTMEFGYSSNSPSTHRSYSYRPYSYRHFAPPTTPCSTDVCDSDYAPSRRMTSVATAKGYTSDLNYDSEPVPPPPTPRSQYLSAEENYESCPPSPYTERSYSHHLYPPPPSPCTDSS

SEQ ID NO: 114 - protein, 784 aa, synthetic construct
  REGION 1..784: note = 1C11-CAR amino acid sequence
MALPVTALLLPLALLLHAARPEVQLVESGGGLVQPGGSLRLSCAASGRTLSRYAMGWFRQAPGKGRELVAAISRTGGSTYYPDSVEGRFTISRDNAKRMVYLQMNSLRAEDTAVYYCAADLYYGPIITEGNYDYWGQGTQVTVSSTTTPAPRPPTPAPTIASQPLSLRPEACRPAAGGAVHTRGLDFACDIYIWAPLAGTCGVLLLSLVITLYCKRGRKKLLYIFKQPFMRPVQTTQEEDGCSCRFPEEEEGGCELRVKFSRSADAPAYQQGQNQLYNELNLGRREEYDVLDKRRGRDPEMGGKPRRKNPQEGLYNELQKDKMAEAYSEIGMKGERRRGKGHDGLYQGLSTATKDTYDALHMQALPPREGRGSLLTCGDVEENPGPMGAVLRSLLACSFCVLLRAEQKLISEEDLEPPTCSPQQFTCFTGEIDCIPVAWRCDGFTECEDHSDELNCPVCSESQFQCASGQCIDGALRCNGDANCQDKSDEKNCEVLCLIDQFRCANGQCIGKHKKCDHNVDCSDKSDELDCYPTEEPAPQATNTVGSVIGVIVTIFVSGTVYFICQRMLCPRMKGDGETMTNDYVVHGPASVPLGYVPHPSSLSGSLPGMSRGKSMISSLSIMGGSSGPPYDRAHVTGASSSSSSSTKGTYFPAILNPPPSPATERSHYTMEFGYSSNSPSTHRSYSYRPYSYRHFAPPTTPCSTDVCDSDYAPSRRMTSVATAKGYTSDLNYDSEPVPPPPTPRSQYLSAEENYESCPPSPYTERSYSHHLYPPPPSPCTDSS

SEQ ID NO: 115 - protein, 784 aa, synthetic construct
  REGION 1..784: note = 1D12-CAR amino acid sequence
MALPVTALLLPLALLLHAARPEVQLVESGGGLVQPGGSLRLSCAASGRTLSPYAMGWFRQAPGKGRELVAAISRTGGSTYYPDSVEGRFTISRDNAKRMVYLQMNSLRAEDTAVYYCAADLYYGPIITEGNYNYWGQGTQVTVSSTTTPAPRPPTPAPTIASQPLSLRPEACRPAAGGAVHTRGLDFACDIYIWAPLAGTCGVLLLSLVITLYCKRGRKKLLYIFKQPFMRPVQTTQEEDGCSCRFPEEEEGGCELRVKFSRSADAPAYQQGQNQLYNELNLGRREEYDVLDKRRGRDPEMGGKPRRKNPQEGLYNELQKDKMAEAYSEIGMKGERRRGKGHDGLYQGLSTATKDTYDALHMQALPPREGRGSLLTCGDVEENPGPMGAVLRSLLACSFCVLLRAEQKLISEEDLEPPTCSPQQFTCFTGEIDCIPVAWRCDGFTECEDHSDELNCPVCSESQFQCASGQCIDGALRCNGDANCQDKSDEKNCEVLCLIDQFRCANGQCIGKHKKCDHNVDCSDKSDELDCYPTEEPAPQATNTVGSVIGVIVTIFVSGTVYFICQRMLCPRMKGDGETMTNDYVVHGPASVPLGYVPHPSSLSGSLPGMSRGKSMISSLSIMGGSSGPPYDRAHVTGASSSSSSSTKGTYFPAILNPPPSPATERSHYTMEFGYSSNSPSTHRSYSYRPYSYRHFAPPTTPCSTDVCDSDYAPSRRMTSVATAKGYTSDLNYDSEPVPPPPTPRSQYLSAEENYESCPPSPYTERSYSHHLYPPPPSPCTDSS

SEQ ID NO: 116 - protein, 781 aa, synthetic construct
  REGION 1..781: note = 2F9-CAR amino acid sequence
MALPVTALLLPLALLLHAARPEVQLVESGGGLVQPGGSLRLSCAASGRILSRYAMGWFRQAPGKGRELVATISARGSSTYYPDSVEGRFTISRDNAKRMVYLQMNSLRAEDTAVYYCAANDITYTQATYDYWGQGTQVTVSSTTTPAPRPPTPAPTIASQPLSLRPEACRPAAGGAVHTRGLDFACDIYIWAPLAGTCGVLLLSLVITLYCKRGRKKLLYIFKQPFMRPVQTTQEEDGCSCRFPEEEEGGCELRVKFSRSADAPAYQQGQNQLYNELNLGRREEYDVLDKRRGRDPEMGGKPRRKNPQEGLYNELQKDKMAEAYSEIGMKGERRRGKGHDGLYQGLSTATKDTYDALHMQALPPREGRGSLLTCGDVEENPGPMGAVLRSLLACSFCVLLRAEQKLISEEDLEPPTCSPQQFTCFTGEIDCIPVAWRCDGFTECEDHSDELNCPVCSESQFQCASGQCIDGALRCNGDANCQDKSDEKNCEVLCLIDQFRCANGQCIGKHKKCDHNVDCSDKSDELDCYPTEEPAPQATNTVGSVIGVIVTIFVSGTVYFICQRMLCPRMKGDGETMTNDYVVHGPASVPLGYVPHPSSLSGSLPGMSRGKSMISSLSIMGGSSGPPYDRAHVTGASSSSSSSTKGTYFPAILNPPPSPATERSHYTMEFGYSSNSPSTHRSYSYRPYSYRHFAPPTTPCSTDVCDSDYAPSRRMTSVATAKGYTSDLNYDSEPVPPPPTPRSQYLSAEENYESCPPSPYTERSYSHHLYPPPPSPCTDSS

SEQ ID NO: 117 - protein, 784 aa, synthetic construct
  REGION 1..784: note = 3-CAR amino acid sequence
MALPVTALLLPLALLLHAARPEVQLVESGGGLVQPGGSLRLSCAASGRTFSSYAMGWFRQAPGKGRELVAAISRTGGSTYYPDSVEGRFTISRDNAKRMVYLQMNSLRAEDTAVYYCAADLYYGPIITEGNYDYWGQGTQVTVSSTTTPAPRPPTPAPTIASQPLSLRPEACRPAAGGAVHTRGLDFACDIYIWAPLAGTCGVLLLSLVITLYCKRGRKKLLYIFKQPFMRPVQTTQEEDGCSCRFPEEEEGGCELRVKFSRSADAPAYQQGQNQLYNELNLGRREEYDVLDKRRGRDPEMGGKPRRKNPQEGLYNELQKDKMAEAYSEIGMKGERRRGKGHDGLYQGLSTATKDTYDALHMQALPPREGRGSLLTCGDVEENPGPMGAVLRSLLACSFCVLLRAEQKLISEEDLEPPTCSPQQFTCFTGEIDCIPVAWRCDGFTECEDHSDELNCPVCSESQFQCASGQCIDGALRCNGDANCQDKSDEKNCEVLCLIDQFRCANGQCIGKHKKCDHNVDCSDKSDELDCYPTEEPAPQATNTVGSVIGVIVTIFVSGTVYFICQRMLCPRMKGDGETMTNDYVVHGPASVPLGYVPHPSSLSGSLPGMSRGKSMISSLSIMGGSSGPPYDRAHVTGASSSSSSSTKGTYFPAILNPPPSPATERSHYTMEFGYSSNSPSTHRSYSYRPYSYRHFAPPTTPCSTDVCDSDYAPSRRMTSVATAKGYTSDLNYDSEPVPPPPTPRSQYLSAEENYESCPPSPYTERSYSHHLYPPPPSPCTDSS

SEQ ID NO: 118 - protein, 784 aa, synthetic construct
  REGION 1..784: note = 4-CAR amino acid sequence
MALPVTALLLPLALLLHAARPEVQLVESGGGLVQPGGSLRLSCAASGSIFSTYAMGWFRQAPGKGRELVAAISRTGGSTYYPDSVEGRFTISRDNAKRMVYLQMNSLRAEDTAVYYCAADLYYGPIITEGNYDYWGQGTQVTVSSTTTPAPRPPTPAPTIASQPLSLRPEACRPAAGGAVHTRGLDFACDIYIWAPLAGTCGVLLLSLVITLYCKRGRKKLLYIFKQPFMRPVQTTQEEDGCSCRFPEEEEGGCELRVKFSRSADAPAYQQGQNQLYNELNLGRREEYDVLDKRRGRDPEMGGKPRRKNPQEGLYNELQKDKMAEAYSEIGMKGERRRGKGHDGLYQGLSTATKDTYDALHMQALPPREGRGSLLTCGDVEENPGPMGAVLRSLLACSFCVLLRAEQKLISEEDLEPPTCSPQQFTCFTGEIDCIPVAWRCDGFTECEDHSDELNCPVCSESQFQCASGQCIDGALRCNGDANCQDKSDEKNCEVLCLIDQFRCANGQCIGKHKKCDHNVDCSDKSDELDCYPTEEPAPQATNTVGSVIGVIVTIFVSGTVYFICQRMLCPRMKGDGETMTNDYVVHGPASVPLGYVPHPSSLSGSLPGMSRGKSMISSLSIMGGSSGPPYDRAHVTGASSSSSSSTKGTYFPAILNPPPSPATERSHYTMEFGYSSNSPSTHRSYSYRPYSYRHFAPPTTPCSTDVCDSDYAPSRRMTSVATAKGYTSDLNYDSEPVPPPPTPRSQYLSAEENYESCPPSPYTERSYSHHLYPPPPSPCTDSS

SEQ ID NO: 119 - protein, 784 aa, synthetic construct
  REGION 1..784: note = 7-CAR amino acid sequence
MALPVTALLLPLALLLHAARPEVQLVESGGGLVQPGGSLRLSCAASGRTLSRYAMGWFRQAPGKGRELVAAISRTGGSTYYPDSVEGRFTISRDNAKRMVYLQMNSLRAEDTAVYYCAADLYYGPIITEGNYNYWGQGTQVTVSSTTTPAPRPPTPAPTIASQPLSLRPEACRPAAGGAVHTRGLDFACDIYIWAPLAGTCGVLLLSLVITLYCKRGRKKLLYIFKQPFMRPVQTTQEEDGCSCRFPEEEEGGCELRVKFSRSADAPAYQQGQNQLYNELNLGRREEYDVLDKRRGRDPEMGGKPRRKNPQEGLYNELQKDKMAEAYSEIGMKGERRRGKGHDGLYQGLSTATKDTYDALHMQALPPREGRGSLLTCGDVEENPGPMGAVLRSLLACSFCVLLRAEQKLISEEDLEPPTCSPQQFTCFTGEIDCIPVAWRCDGFTECEDHSDELNCPVCSESQFQCASGQCIDGALRCNGDANCQDKSDEKNCEVLCLIDQFRCANGQCIGKHKKCDHNVDCSDKSDELDCYPTEEPAPQATNTVGSVIGVIVTIFVSGTVYFICQRMLCPRMKGDGETMTNDYVVHGPASVPLGYVPHPSSLSGSLPGMSRGKSMISSLSIMGGSSGPPYDRAHVTGASSSSSSSTKGTYFPAILNPPPSPATERSHYTMEFGYSSNSPSTHRSYSYRPYSYRHFAPPTTPCSTDVCDSDYAPSRRMTSVATAKGYTSDLNYDSEPVPPPPTPRSQYLSAEENYESCPPSPYTERSYSHHLYPPPPSPCTDSS

SEQ ID NO: 120 - protein, 784 aa, synthetic construct
  REGION 1..784: note = 8-CAR amino acid sequence
MALPVTALLLPLALLLHAARPEVQLVESGGGLVQPGGSLRLSCAASGDTLSRYAMGWFRQAPGKGRELVAAISRTGGSTYYPDSVEGRFTISRDNAKRMVYLQMNSLRAEDTAVYYCAADLYYGPIITEGNYNYWGQGTQVTVSSTTTPAPRPPTPAPTIASQPLSLRPEACRPAAGGAVHTRGLDFACDIYIWAPLAGTCGVLLLSLVITLYCKRGRKKLLYIFKQPFMRPVQTTQEEDGCSCRFPEEEEGGCELRVKFSRSADAPAYQQGQNQLYNELNLGRREEYDVLDKRRGRDPEMGGKPRRKNPQEGLYNELQKDKMAEAYSEIGMKGERRRGKGHDGLYQGLSTATKDTYDALHMQALPPREGRGSLLTCGDVEENPGPMGAVLRSLLACSFCVLLRAEQKLISEEDLEPPTCSPQQFTCFTGEIDCIPVAWRCDGFTECEDHSDELNCPVCSESQFQCASGQCIDGALRCNGDANCQDKSDEKNCEVLCLIDQFRCANGQCIGKHKKCDHNVDCSDKSDELDCYPTEEPAPQATNTVGSVIGVIVTIFVSGTVYFICQRMLCPRMKGDGETMTNDYVVHGPASVPLGYVPHPSSLSGSLPGMSRGKSMISSLSIMGGSSGPPYDRAHVTGASSSSSSSTKGTYFPAILNPPPSPATERSHYTMEFGYSSNSPSTHRSYSYRPYSYRHFAPPTTPCSTDVCDSDYAPSRRMTSVATAKGYTSDLNYDSEPVPPPPTPRSQYLSAEENYESCPPSPYTERSYSHHLYPPPPSPCTDSS

SEQ ID NO: 121 - protein, 781 aa, synthetic construct
  REGION 1..781: note = 15-CAR amino acid sequence
MALPVTALLLPLALLLHAARPEVQLVESGGGLVQPGGSLRLSCAASGLIFSRYYMGWFRQAPGKGRELVAGITRSGGGTYYPDSVEGRFTISRDNAKRMVYLQMNSLRAEDTAVYYCAAEPAGYYQENYDYWGQGTQVTVSSTTTPAPRPPTPAPTIASQPLSLRPEACRPAAGGAVHTRGLDFACDIYIWAPLAGTCGVLLLSLVITLYCKRGRKKLLYIFKQPFMRPVQTTQEEDGCSCRFPEEEEGGCELRVKFSRSADAPAYQQGQNQLYNELNLGRREEYDVLDKRRGRDPEMGGKPRRKNPQEGLYNELQKDKMAEAYSEIGMKGERRRGKGHDGLYQGLSTATKDTYDALHMQALPPREGRGSLLTCGDVEENPGPMGAVLRSLLACSFCVLLRAEQKLISEEDLEPPTCSPQQFTCFTGEIDCIPVAWRCDGFTECEDHSDELNCPVCSESQFQCASGQCIDGALRCNGDANCQDKSDEKNCEVLCLIDQFRCANGQCIGKHKKCDHNVDCSDKSDELDCYPTEEPAPQATNTVGSVIGVIVTIFVSGTVYFICQRMLCPRMKGDGETMTNDYVVHGPASVPLGYVPHPSSLSGSLPGMSRGKSMISSLSIMGGSSGPPYDRAHVTGASSSSSSSTKGTYFPAILNPPPSPATERSHYTMEFGYSSNSPSTHRSYSYRPYSYRHFAPPTTPCSTDVCDSDYAPSRRMTSVATAKGYTSDLNYDSEPVPPPPTPRSQYLSAEENYESCPPSPYTERSYSHHLYPPPPSPCTDSS

SEQ ID NO: 122 - protein, 780 aa, synthetic construct
  REGION 1..780: note = 17-CAR amino acid sequence
MALPVTALLLPLALLLHAARPEVQLVESGGGLVQPGGSLRLSCAASGLIFSNDYMGWFRQAPGKGRELVATISTRGGTYYPHNVEGRFIIIRDNDKRMVYLLMNSLRAEDTAVYYCAADSIIGYATEYYYCCQGSKVTVSSTTTPAPRPPTPAPTIASQPLSLRPEACRPAAGGAVHTRGLDFACDIYIWAPLAGTCGVLLLSLVITLYCKRGRKKLLYIFKQPFMRPVQTTQEEDGCSCRFPEEEEGGCELRVKFSRSADAPAYQQGQNQLYNELNLGRREEYDVLDKRRGRDPEMGGKPRRKNPQEGLYNELQKDKMAEAYSEIGMKGERRRGKGHDGLYQGLSTATKDTYDALHMQALPPREGRGSLLTCGDVEENPGPMGAVLRSLLACSFCVLLRAEQKLISEEDLEPPTCSPQQFTCFTGEIDCIPVAWRCDGFTECEDHSDELNCPVCSESQFQCASGQCIDGALRCNGDANCQDKSDEKNCEVLCLIDQFRCANGQCIGKHKKCDHNVDCSDKSDELDCYPTEEPAPQATNTVGSVIGVIVTIFVSGTVYFICQRMLCPRMKGDGETMTNDYVVHGPASVPLGYVPHPSSLSGSLPGMSRGKSMISSLSIMGGSSGPPYDRAHVTGASSSSSSSTKGTYFPAILNPPPSPATERSHYTMEFGYSSNSPSTHRSYSYRPYSYRHFAPPTTPCSTDVCDSDYAPSRRMTSVATAKGYTSDLNYDSEPVPPPPTPRSQYLSAEENYESCPPSPYTERSYSHHLYPPPPSPCTDSS

SEQ ID NO: 123 - protein, 781 aa, synthetic construct
  REGION 1..781: note = 24-CAR amino acid sequence
MALPVTALLLPLALLLHAARPEVQLVESGGGLVQPGGSLRLSCAASGRILSRYAMGWFRQAPGKGRELVATISASGGTTYYPDSVEGRFTISRDNAKRMVYLQMNSLRAEDTAVYYCAAADIYSSDADYNYWGQGTQVTVSSTTTPAPRPPTPAPTIASQPLSLRPEACRPAAGGAVHTRGLDFACDIYIWAPLAGTCGVLLLSLVITLYCKRGRKKLLYIFKQPFMRPVQTTQEEDGCSCRFPEEEEGGCELRVKFSRSADAPAYQQGQNQLYNELNLGRREEYDVLDKRRGRDPEMGGKPRRKNPQEGLYNELQKDKMAEAYSEIGMKGERRRGKGHDGLYQGLSTATKDTYDALHMQALPPREGRGSLLTCGDVEENPGPMGAVLRSLLACSFCVLLRAEQKLISEEDLEPPTCSPQQFTCFTGEIDCIPVAWRCDGFTECEDHSDELNCPVCSESQFQCASGQCIDGALRCNGDANCQDKSDEKNCEVLCLIDQFRCANGQCIGKHKKCDHNVDCSDKSDELDCYPTEEPAPQATNTVGSVIGVIVTIFVSGTVYFICQRMLCPRMKGDGETMTNDYVVHGPASVPLGYVPHPSSLSGSLPGMSRGKSMISSLSIMGGSSGPPYDRAHVTGASSSSSSSTKGTYFPAILNPPPSPATERSHYTMEFGYSSNSPSTHRSYSYRPYSYRHFAPPTTPCSTDVCDSDYAPSRRMTSVATAKGYTSDLNYDSEPVPPPPTPRSQYLSAEENYESCPPSPYTERSYSHHLYPPPPSPCTDSS

SEQ ID NO: 124 - protein, 784 aa, synthetic construct
  REGION 1..784: note = 29-CAR amino acid sequence
MALPVTALLLPLALLLHAARPEVQLVESGGGLVQPGGSLRLSCAASGNTFSSYAMGWFRQAPGKGRELVAAISRTGGSTYYPDSVEGRFTISRDNAKRMVYLHMNSLRAEDTAVYYCAADLYYGPIITEGNYNYWGQGTQVTVSSTTTPAPRPPTPAPTIASQPLSLRPEACRPAAGGAVHTRGLDFACDIYIWAPLAGTCGVLLLSLVITLYCKRGRKKLLYIFKQPFMRPVQTTQEEDGCSCRFPEEEEGGCELRVKFSRSADAPAYQQGQNQLYNELNLGRREEYDVLDKRRGRDPEMGGKPRRKNPQEGLYNELQKDKMAEAYSEIGMKGERRRGKGHDGLYQGLSTATKDTYDALHMQALPPREGRGSLLTCGDVEENPGPMGAVLRSLLACSFCVLLRAEQKLISEEDLEPPTCSPQQFTCFTGEIDCIPVAWRCDGFTECEDHSDELNCPVCSESQFQCASGQCIDGALRCNGDANCQDKSDEKNCEVLCLIDQFRCANGQCIGKHKKCDHNVDCSDKSDELDCYPTEEPAPQATNTVGSVIGVIVTIFVSGTVYFICQRMLCPRMKGDGETMTNDYVVHGPASVPLGYVPHPSSLSGSLPGMSRGKSMISSLSIMGGSSGPPYDRAHVTGASSSSSSSTKGTYFPAILNPPPSPATERSHYTMEFGYSSNSPSTHRSYSYRPYSYRHFAPPTTPCSTDVCDSDYAPSRRMTSVATAKGYTSDLNYDSEPVPPPPTPRSQYLSAEENYESCPPSPYTERSYSHHLYPPPPSPCTDSS

SEQ ID NO: 125 - protein, 235 aa, synthetic construct
  REGION 1..235: note = Fc sequence
AAAEPKSCDKTHTCPPCPAPELLGGPSVFLFPPKPKDTLMISRTPEVTCVVVDVSHEDPEVKFNWYVDGVEVHNAKTKPREEQYNSTYRVVSVLTVLHQDWLNGKEYKCKVSNKALPAPIEKTISKAKGQPREPQVYTLPPSRDELTKNQVSLTCLVKGFYPSDIAVEWESNGQPENNYKTTPPVLDSDGSFFLYSKLTVDKSRWQQGNVFSCSVMHEALHNHYTQKSLSLSPGK

SEQ ID NO: 126 - protein, 9 aa, synthetic construct
  REGION 1..9: note = mouse AFP158 peptide
FMNRFIYEV

SEQ ID NO: 127 - DNA, 207 bp, synthetic construct
  misc_feature 1..207: note = CD8 hinge region and transmembrane domain nuleotide
  source 1..207: mol_type = other DNA
accacgacgccagcgccgcgaccaccaacaccggcgcccaccatcgcgtcgcagcccctgtccctgcgcccagaggcgtgccggccagcggcggggggcgcagtgcacacgagggggctggacttcgcctgtgatatctacatctgggcgcccttggccgggacttgtggggtccttctcctgtcactggttatcaccctttactgc

SEQ ID NO: 128 - protein, 69 aa, synthetic construct
  REGION 1..69: note = CD8 hinge region and transmembrane domain
TTTPAPRPPTPAPTIASQPLSLRPEACRPAAGGAVHTRGLDFACDIYIWAPLAGTCGVLLLSLVITLYC

SEQ ID NO: 129 - DNA, 123 bp, synthetic construct
  misc_feature 1..123: note = CD28 intracellular domain nucleotide
  source 1..123: mol_type = other DNA
aggagtaagaggagcaggctcctgcacagtgactacatgaacatgactccccgccgccccgggcccacccgcaagcattaccagccctatgccccaccacgcgacttcgcagcctatcgctcc

SEQ ID NO: 130 - protein, 41 aa, synthetic construct
  REGION 1..41: note = CD28 intracellular domain
RSKRSRLLHSDYMNMTPRRPGPTRKHYQPYAPPRDFAAYRS

SEQ ID NO: 131 - DNA, 126 bp, synthetic construct
  misc_feature 1..126: note = 41BB intracellular domain nucleotide
  source 1..126: mol_type = other DNA
aaacggggcagaaagaaactcctgtatatattcaaacaaccatttatgagaccagtacaaactactcaagaggaagatggctgtagctgccgatttccagaagaagaagaaggaggatgtgaactg

SEQ ID NO: 132 - protein, 42 aa, synthetic construct
  REGION 1..42: note = 41BB intracellular domain
KRGRKKLLYIFKQPFMRPVQTTQEEDGCSCRFPEEEEGGCEL

SEQ ID NO: 133 - DNA, 339 bp, synthetic construct
  misc_feature 1..339: note = CD3zeta nucleotide
  source 1..339: mol_type = other DNA
agagtgaagttcagcaggagcgcagacgcccccgcgtaccagcagggccagaaccagctctataacgagctcaatctaggacgaagagaggagtacgatgttttggacaagagacgtggccgggaccctgagatggggggaaagccgagaaggaagaaccctcaggaaggcctgtacaatgaactgcagaaagataagatggcggaggcctacagtgagattgggatgaaaggcgagcgccggaggggcaaggggcacgatggcctttaccagggtctcagtacagccaccaaggacacctacgacgcccttcacatgcaggccctgccccctcgctaa

SEQ ID NO: 134 - protein, 112 aa, synthetic construct
  REGION 1..112: note = CD3zeta
RVKFSRSADAPAYQQGQNQLYNELNLGRREEYDVLDKRRGRDPEMGGKPRRKNPQEGLYNELQKDKMAEAYSEIGMKGERRRGKGHDGLYQGLSTATKDTYDALHMQALPPR

SEQ ID NO: 135 - DNA, 54 bp, synthetic construct
  misc_feature 1..54: note = 2A nucleotide
  source 1..54: mol_type = other DNA
gagggcagaggaagtcttctaacatgcggtgacgtggaggagaatcccggccct

SEQ ID NO: 136 - protein, 18 aa, synthetic construct
  REGION 1..18: note = 2A
EGRGSLLTCGDVEENPGP

SEQ ID NO: 137 - DNA, 1167 bp, synthetic construct
  misc_feature 1..1167: note = L6 nucleotide
  source 1..1167: mol_type = other DNA
atgggggccgtcctgaggagcctcctggcctgcagcttctgtgtgctcctgagagcggaacctccaacatgttctcctcagcagtttacttgtttcacgggggaaattgactgtatccctgtggcttggcggtgcgatgggtttactgaatgtgaagaccacagtgatgaactcaattgtcctgtatgctcagagtcccagttccagtgtgccagtgggcagtgtattgatggtgccctccgatgcaatggagatgcaaactgccaggacaaatcagatgagaagaactgtgaagtgctttgtttaattgatcagttccgctgtgccaatggtcagtgcattggaaagcacaagaagtgtgatcataatgtggattgcagtgacaagtcagatgaactggattgttatccgactgaagaaccagcaccacaggccaccaatacagttggttctgttattggcgtaattgtcaccatttttgtgtctggaactgtatactttatctgccagaggatgttgtgtccacgtatgaagggagatggggaaactatgactaatgactatgtagttcatggaccagcttctgtgcctcttggttatgtgccacacccaagttctttgtcaggatctcttccaggaatgtctcgaggtaaatcaatgatcagctccctcagtatcatggggggaagcagtggacccccctatgaccgagcccatgttacaggagcatcatcaagtagttcttcaagcaccaaaggcacttacttccctgcaattttgaaccctccaccatccccagccacagagcgatcacattacactatggaatttggatattcttcaaacagtccttccactcataggtcatacagctacaggccatatagctaccggcactttgcaccccccaccacaccctgcagcacagatgtttgtgacagtgactatgctcctagtcggagaatgacctcagtggcaacagccaagggctataccagtgacttgaactatgattcagaacctgtgcccccacctcccacaccccgaagccaatacttgtcagcagaggagaactatgaaagctgcccaccttctccatacacagagaggagctattctcatcacctctacccaccgccaccctctccctgtacagactcctcctga

SEQ ID NO: 138 - protein, 370 aa, synthetic construct
  REGION 1..370: note = L6
GEPPTCSPQQFTCFTGEIDCIPVAWRCDGFTECEDHSDELNCPVCSESQFQCASGQCIDGALRCNGDANCQDKSDEKNCEVLCLIDQFRCANGQCIGKHKKCDHNVDCSDKSDELDCYPTEEPAPQATNTVGSVIGVIVTIFVSGTVYFICQRMLCPRMKGDGETMTNDYVVHGPASVPLGYVPHPSSLSGSLPGMSRGKSMISSLSIMGGSSGPPYDRAHVTGASSSSSSSTKGTYFPAILNPPPSPATERSHYTMEFGYSSNSPSTHRSYSYRPYSYRHFAPPTTPCSTDVCDSDYAPSRRMTSVATAKGYTSDLNYDSEPVPPPPTPRSQYLSAEENYESCPPSPYTERSYSHHLYPPPPSPCTDSS

SEQ ID NO: 139 - DNA, 804 bp, synthetic construct
  misc_feature 1..804: note = TL6 nucleotide
  source 1..804: mol_type = other DNA
atgggggccgtcctgaggagcctcctggcctgcagcttctgtgtgctcctgagagcgccagcaccacaggccaccaatacagttggttctgttattggcgtaattgtcaccatttttgtgtctggaactgtatactttatctgccagaggatgttgtgtccacgtatgaagggagatggggaaactatgactaatgactatgtagttcatggaccagcttctgtgcctcttggttatgtgccacacccaagttctttgtcaggatctcttccaggaatgtctcgaggtaaatcaatgatcagctccctcagtatcatggggggaagcagtggacccccctatgaccgagcccatgttacaggagcatcatcaagtagttcttcaagcaccaaaggcacttacttccctgcaattttgaaccctccaccatccccagccacagagcgatcacattacactatggaatttggatattcttcaaacagtccttccactcataggtcatacagctacaggccatatagctaccggcactttgcaccccccaccacaccctgcagcacagatgtttgtgacagtgactatgctcctagtcggagaatgacctcagtggcaacagccaagggctataccagtgacttgaactatgattcagaacctgtgcccccacctcccacaccccgaagccaatacttgtcagcagaggagaactatgaaagctgcccaccttctccatacacagagaggagctattctcatcacctctacccaccgccaccctctccctgtacagactcctcctga

SEQ ID NO: 140 - protein, 243 aa, synthetic construct
  REGION 1..243: note = TL6
TNTVGSVIGVIVTIFVSGTVYFICQRMLCPRMKGDGETMTNDYVVHGPASVPLGYVPHPSSLSGSLPGMSRGKSMISSLSIMGGSSGPPYDRAHVTGASSSSSSSTKGTYFPAILNPPPSPATERSHYTMEFGYSSNSPSTHRSYSYRPYSYRHFAPPTTPCSTDVCDSDYAPSRRMTSVATAKGYTSDLNYDSEPVPPPPTPRSQYLSAEENYESCPPSPYTERSYSHHLYPPPPSPCTDSS

SEQ ID NO: 141 - DNA, 1089 bp, synthetic construct
  misc_feature 1..1089: note = L5 nucleotide
  source 1..1089: mol_type = other DNA
ggagagccgcccacctgctccccggaccagtttgcatgtgccacaggggagatcgactgtatccccggggcctggcgctgtgacggctttcccgagtgcgatgaccagagcgacgaggagggctgccccgtgtgctccgccgcccagttcccctgcgcgcggggtcagtgtgtggacctgcgcctgcgctgcgacggcgaggcagactgtcaggaccgctcagacgaggcggactgtgacgccatctgcctgcccaaccagttccggtgtgcgagcggccagtgtgtcctcatcaaacagcagtgcgactccttccccgactgtatcgacggctccgacgagctcatgtgtgaaatcaccaagccgccctcagacgacagcccggcccacagcagtgccatcgggcccgtcattggcatcatcctctctctcttcgtcatgggtggtgtctattttgtgtgccagcgcgtggtgtgccagcgctatgcgggggccaacgggcccttcccgcacgagtatgtcagcgggaccccgcacgtgcccctcaatttcatagccccgggcggttcccagcatggccccttcacaggcatcgcatgcggaaagtccatgatgagctccgtgagcctgatggggggccggggcggggtgcccctctacgaccggaaccacgtcacaggggcctcgtccagcagctcgtccagcacgaaggccacgctgtacccgccgatcctgaacccgccgccctccccggccacggacccctccctgtacaacatggacatgttctactcttcaaacattccggccactgcgagaccgtacaggccctacatcattcgaggaatggcgcccccgacgacgccctgcagcaccgacgtgtgtgacagcgactacagcgccagccgctggaaggccagcaagtactacctggatttgaactcggactcagacccctatccacccccacccacgccccacagccagtacctgtcggcggaggacagctgcccgccctcgcccgccaccgagaggagctacttccatctcttcccgccccctccgtccccctgcacggactcatcctga

SEQ ID NO: 142 - protein, 362 aa, synthetic construct
  REGION 1..362: note = L5
GEPPTCSPDQFACATGEIDCIPGAWRCDGFPECDDQSDEEGCPVCSAAQFPCARGQCVDLRLRCDGEADCQDRSDEADCDAICLPNQFRCASGQCVLIKQQCDSFPDCIDGSDELMCEITKPPSDDSPAHSSAIGPVIGIILSLFVMGGVYFVCQRVVCQRYAGANGPFPHEYVSGTPHVPLNFIAPGGSQHGPFTGIACGKSMMSSVSLMGGRGGVPLYDRNHVTGASSSSSSSTKATLYPPILNPPPSPATDPSLYNMDMFYSSNIPATARPYRPYIIRGMAPPTTPCSTDVCDSDYSASRWKASKYYLDLNSDSDPYPPPPTPHSQYLSAEDSCPPSPATERSYFHLFPPPPSPCTDSS

SEQ ID NO: 143 - DNA, 696 bp, synthetic construct
  misc_feature 1..696: note = TL5 nucleotide
  source 1..696: mol_type = other DNA
agtgccatcgggcccgtcattggcatcatcctctctctcttcgtcatgggtggtgtctattttgtgtgccagcgcgtggtgtgccagcgctatgcgggggccaacgggcccttcccgcacgagtatgtcagcgggaccccgcacgtgcccctcaatttcatagccccgggcggttcccagcatggccccttcacaggcatcgcatgcggaaagtccatgatgagctccgtgagcctgatggggggccggggcggggtgcccctctacgaccggaaccacgtcacaggggcctcgtccagcagctcgtccagcacgaaggccacgctgtacccgccgatcctgaacccgccgccctccccggccacggacccctccctgtacaacatggacatgttctactcttcaaacattccggccactgcgagaccgtacaggccctacatcattcgaggaatggcgcccccgacgacgccctgcagcaccgacgtgtgtgacagcgactacagcgccagccgctggaaggccagcaagtactacctggatttgaactcggactcagacccctatccacccccacccacgccccacagccagtacctgtcggcggaggacagctgcccgccctcgcccgccaccgagaggagctacttccatctcttcccgccccctccgtccccctgcacggactcatcctga

SEQ ID NO: 144 - protein, 231 aa, synthetic construct
  REGION 1..231: note = TL5
SAIGPVIGIILSLFVMGGVYFVCQRVVCQRYAGANGPFPHEYVSGTPHVPLNFIAPGGSQHGPFTGIACGKSMMSSVSLMGGRGGVPLYDRNHVTGASSSSSSSTKATLYPPILNPPPSPATDPSLYNMDMFYSSNIPATARPYRPYIIRGMAPPTTPCSTDVCDSDYSASRWKASKYYLDLNSDSDPYPPPPTPHSQYLSAEDSCPPSPATERSYFHLFPPPPSPCTDSS

SEQ ID NO: 145 - DNA, 578 bp, synthetic construct
  misc_feature 1..578: note = IRES sequence
  source 1..578: mol_type = other DNA
tccctcccccccccctaacgttactggccgaagccgcttggaataaggccggtgtgcgtttgtctatatgttattttccaccatattgccgtcttttggcaatgtgagggcccggaaacctggccctgtcttcttgacgagcattcctaggggtctttcccctctcgccaaaggaatgcaaggtctgttgaatgtcgtgaaggaagcagttcctctggaagcttcttgaagacaaacaacgtctgtagcgaccctttgcaggcagcggaaccccccacctggcgacaggtgcctctgcggccaaaagccacgtgtataagatacacctgcaaaggcggcacaaccccagtgccacgttgtgagttggatagttgtggaaagagtcaaatggctctcctcaagcgtattcaacaaggggctgaaggatgcccagaaggtaccccattgtatgggatctgatctggggcctcggtgcacatgctttacatgtgtttagtcgaggttaaaaaaacgtctaggccccccgaaccacggggacgtggttttcctttgaaaaacacgatgataatatggccaca

SEQ ID NO: 146 - DNA, 63 bp, synthetic construct
  misc_feature 1..63: note = leader nucleotide sequence
  source 1..63: mol_type = other DNA
atggctctgcctgtgaccgctctgctgctgcctctggctctgctgctgcacgccgcaagacct

SEQ ID NO: 147 - protein, 45 aa, synthetic construct
  REGION 1..45: note = CD8 hinge region sequence
TTTPAPRPPTPAPTIASQPLSLRPEACRPAAGGAVHTRGLDFACD

SEQ ID NO: 148 - DNA, 135 bp, synthetic construct
  misc_feature 1..135: note = CD8 hinge region nucleotide sequence
  source 1..135: mol_type = other DNA
accacgacgccagcgccgcgaccaccaacaccggcgcccaccatcgcgtcgcagcccctgtccctgcgcccagaggcgtgccggccagcggcggggggcgcagtgcacacgagggggctggacttcgcctgtgat

SEQ ID NO: 149 - protein, 24 aa, synthetic construct
  REGION 1..24: note = CD8 transmembrane sequence
IYIWAPLAGTCGVLLLSLVITLYC

SEQ ID NO: 150 - DNA, 72 bp, synthetic construct
  misc_feature 1..72: note = CD8 transmembrane nucleotide sequence
  source 1..72: mol_type = other DNA
atctacatctgggcgcccttggccgggacttgtggggtccttctcctgtcactggttatcaccctttactgc